European Patent Application EP 4 265 722 A2, published October 25, 2023. Title: PROCESSO PARA CONSTRUÇÃO DE UM ÚNICO VETOR COMPREENDENDO CAS9 E SGRNA PARA MODIFICAÇÕES DO GENOMA DE MICOBACTÉRIAS. Applicant: INSTITUTO BUTANTAN. The sequence listing filed with the application follows.

SEQUENCE LISTING (21 sequences)

SEQ ID NO: 1 - DNA, 33 bp, Streptococcus pyogenes M1
tggcatccgtggcgcggccgcagaaatattgga

SEQ ID NO: 2 - DNA, 31 bp, Streptococcus pyogenes M1
tcgctggcatcgataaaggggacctctaggg

SEQ ID NO: 3 - DNA, 28 bp, Escherichia coli
  misc_feature (26)..(26): n is a, c, g, t or u
tatcgatgccagcgagtcatgaggtnac

SEQ ID NO: 4 - DNA, 26 bp, Escherichia coli
tctacgtagtcgacgcatgcctcgag

SEQ ID NO: 5 - DNA, 39 bp, Streptococcus pyogenes
gcgtcgactacgtagaattcagaaatattggatcgtcgg

SEQ ID NO: 6 - DNA, 53 bp, Streptococcus pyogenes
ctagttaactacgtcgacattctagattaattaaaaaaaagcaccgactcggt

SEQ ID NO: 7 - DNA, 44 bp, Escherichia coli
tagcagctggcggccgctcattgacccttcacctccaggctcag

SEQ ID NO: 8 - DNA, 44 bp, Escherichia coli; identical to SEQ ID NO: 7

SEQ ID NO: 9 - DNA, 24 bp, Mycobacterium bovis
gggagtgcaaacgtccagacagag

SEQ ID NO: 10 - DNA, 24 bp, Mycobacterium bovis
aaacctctgtctggacgtttgcac

SEQ ID NO: 11 - DNA, 24 bp, Mycobacterium bovis
gggagtcggaaagcactgcgaaag

SEQ ID NO: 12 - DNA, 24 bp, Iniciador antisenso crRNA-lysA88-BCG
aaacctttcgcagtgctttccgac

SEQ ID NO: 13 - DNA, 27 bp, Mycobacterium smegmatis
gggatgcaccgtgatccgcgaggccgg

SEQ ID NO: 14 - DNA, 27 bp, Mycobacterium smegmatis
aaacccggcctcgcggatcacggtgca

SEQ ID NO: 15 - DNA, 27 bp, Mycobacterium smegmatis
gggacagatgtccatcgtggatctcgg

SEQ ID NO: 16 - DNA, 27 bp, Mycobacterium smegmatis
aaacccgagatccacgatggacatctg

SEQ ID NO: 17 - DNA, 27 bp, Mycobacterium smegmatis
gggaggttcgcggtgccgacggggtgg

SEQ ID NO: 18 - DNA, 27 bp, Mycobacterium smegmatis
aaacccaccccgtcggcaccgcgaacc

SEQ ID NO: 19 - DNA, 9812 bp, Escherichia coli
  misc_feature (8887)..(8887): n is a, c, g, or t
gctagctatttaattggggaccctagaggtccccttttacgtagaattcagaaatattggatcgtcggcaccgtcacggccgtgggaggcggcacgatccgcgacgtgatgatcggccgcatccccacggtgctgcgcagtgagctctacgccatcccggcgttgatctgtgcgttcgcacgcacaggcccggtgtgagaagggtctctgacgagcgggagaactccctatcagtgatagagtttgtcctccctatcagtgatagataggctctgggagggtcttcgagaagacctgttttagagctagaaatagcaagttaaaataaggctagtccgttatcaacttgaaaaagtggcaccgagtcggtgcttttttttaattaatctagagggaccctagaggtcccctttgctagccaacaaagcgacgttgtgtctcaaaatctctgatgttacattgcacaagataaaaatatatcatcatgaacaataaaactgtctgcttacataaacagtaatacaaggggtgttatgagccatattcaacgggaaacgtcttgctcgaggccgcgattaaattccaacatggatgctgatttatatgggtataaatgggctcgcgataatgtcgggcaatcaggtgcgacaatctatcgcttgtatgggaagccccatgcgccagagttgtttctgaaacatggcaaaggtagcgttgccaatgatgttacagatgagatggtcagactaaactggctgacggaatttatgcctcttccgaccatcaagcattttatccgtactcctgatgatgcatggttactcaccactgcgatccccgggaaaacagcattccaggtattagaagaatatcctgattcaggtgaaaatattgttgatgcgctggcagtgttcctgcgccggttgcattcgattcctgtttgtaattgtccttttaacagcgatcgcgtatttcgtctcgctcaggcgcaatcacgaatgaataacggtttggttgatgcgagtgattttgatgacgagcgtaatggctggcctgttgaacaagtctggaaagaaatgcataatcttttgccattctcaccggattcagtcgtcactcatggtgatttctcacttgataaccttatttttgacgaggggaaattaataggttgtattgatgttggacgagtcggaatcgcagaccgataccaggatcttgccatcctatggaactgcctcggtgagttttctccttcattacagaaacggctttttcaaaaatatggtattgataatcctgatatgaataaattgcagtttcatttgatgctcgatgagtttttctaatcagaattggttaattggttgtaacactggcagagcattacgctgacttgacgggacggcggctttgttgaataaatcgaacttttgctgagttgaaggatcagatcacgcatcttcccgacaacgcagaccgttccgtggcaaagcaaaagttcaaaatcaccaactggtccacctacaacaaagctctcatcaaccgtggctccctcactttctggctggatgatggggcgattcaggcctggtatgagtcagcaacaccttcttcacgaggcagacctcactagttccactgagcgtcagaccccgtagaaaagatcaaaggatcttcttgagatcctttttttctgcgcgtaatctgctgcttgcaaacaaaaaaaccaccgctaccagcggtggtttgtttgccggatcaagagctaccaactctttttccgaaggtaactggcttcagcagagcgcagataccaaatactgtccttctagtgtagccgtagttaggccaccacttcaagaactctgtagcaccgcctacatacctcgctctgctaatcctgttaccagtggctgctgccagtggcgataagtcgtgtcttaccgggttggactcaagacgatagttaccggataaggcgcagcggtcgggctgaacggggggttcgtgcacacagcccagcttggagcgaacgacctacaccgaactgagatacctacagcgtgagcattgagaaagcgccacgcttcccgaagggagaaaggcggacaggtatccggtaagcggcagggtcggaacaggagagcgcacgagggagcttccagggggaaacgcctggtatctttatagtcctgtcgggtttcgccacctctgacttgagcgtcgatttttgtgatgctcgtcaggggggcggagcctatggaaaaacgccagcaacgcggcctttttacggttcctggccttttgctggccttttgctcacatgttctttcctgcgttatcccctgattctgtggataaccgtattaccgcctttgagtgagctgataccgctcgccgcagccgaacgaccgagcgcaacgcgtgagcccaccagctccgtaagttcgggtgctgtgtggctcgtacccgcgcattcaggcggcagggggtctaacgggtctaaggcggcgtgtacggccgccacagcggctcttagcggcccggaaacgtcctcgaaacgacgcatgtgttcctcctggttggtacaggtggttgggggtgctcggctgtcgctggtgtttcatcatcagggctcgacgggagagcgggggagtgtgcagttgtggggtggcccctcagcgaaatatctgacttggagctcgtgtcggaccatacaccggtgattaatcgtggtttattatcaagcgtgagccacgtcgccgacgaatttgagcagctctggctgccgtactggtccctggcaagcgacgatctgctcgaggggatctaccgccaaagccgcgcgtcggccctaggccgccggtacatcgaggcgaacccaacagcgctggcaaacctgctggtcgtggacgtagaccatccagacgcagcgctccgagcgctcagcgcccgggggtcccatccgctgcccaacgcgatcgtgggcaatcgcgccaacggccacgcacacgcagtgtgggcactcaacgcccctgttccacgcaccgaatacgcgcggcgtaagccgctcgcatacatggcggcgtgcgccgaaggccttcggcgcgccgtcgatggcgaccgcagttactcaggcctcatgaccaaaaaccccggccacatcgcctgggaaacggaatggctccactcagatctctacacactcagccacatcgaggccgagctcggcgcgaacatgccaccgccgcgctggcgtcagcagaccacgtacaaagcggctccgacgccgctagggcggaattgcgcactgttcgattccgtcaggttgtgggcctatcttcccgccctcatgcggatctacctgccgacccggaacgtggacggactcggccgcgcgatctatgccgagtgccacgcgcgaaacgccgaatttccgtgcaacgacgtgtgtcccggaccgctaccggacagcgaggtccgcgccatcgccaacagcatttggcgttggatcacaaccaagtcgcgcatttgggcggacgggatcgtggtctacgaggccacactcagtgcgcgccatgcggccatctcgcggaagggcgcagcagcgcgcacggcggcgagcacagttgcgcggcgcgcaaagtccgcgtcagccatggaggcattgctatgagcgacggctacagcgacggctacagcgacggctacaactggcagccgactgtccgcaaaaagcggcgcgtgaccgccgccgaaggcgctcgaatcaccggactatccgaacgccacgtcgtccggctcgtggcgcaggaacgcagcgagtggttcgccgagcaggctgcacgccgcgaacgcatccgcgcctatcacgacgacgagggccactcttggccgcaaacggccaaacatttcgggctgcatctggacaccgttaagcgactcggctatcgggcgaggaaagagcgtgcggcagaacaggaagcggctcaaaaggcccacaacgaagccgacaatccaccgctgttctaacgcaattggggagcgggtgtcgcgggggttccgtggggggttccgttgcaacgggtcggacaggtaaaagtcctggtagacgctagttttctggtttgggccatgcctgtctcgttgcgtgtttcgttgcgtccgttttgaataccagccagacgagacggggttctacgaatcttggtcgataccaagccatttccgctgaatatcgtggagctcaccgccagaatcggtggttgtggtgatgtacgtggcgaactccgttgtagtgcttgtggtggcatccgtggcgcggccgcagaaatattggatcgtcggcaccgtcacggccgtgggaggcggcacgatccgcgacgtgatgatcggccgcatccccacggtgctgcgcagtgagctctacgccatcccggcgttgatctgtgcgttcgcacgcacaggcccggtgtgagaagggtctctgacgagcgggagaactccctatcagtgatagagtttgtcctccctatcagtgatagataggctctgggagtacccgtgtgtacgaccagcacggcatacatcatttcgacgccgagagattcgccgcccgaaatgagcacgatccgggatccggtaccatggacaagaagtacagcatcggcctggacatcggcacgaactcggtgggctgggcggtcatcacggacgagtacaaggtcccctccaagaagttcaaggtcctgggcaacaccgaccggcacagcatcaagaagaacctgatcggcgccctgctgttcgactccggcgagaccgccgaggcgacgcgcctgaagcggaccgcgcggcgccgatacacgcggcgcaagaaccgcatctgctacctgcaggaaatcttctcgaacgagatggccaaggtggacgacagcttcttccaccggctggaggagtccttcctggtggaggaggacaagaagcacgagcgccacccgatcttcggcaacatcgtggacgaggtggcctaccacgagaagtaccccacgatctaccacctgcgcaagaagctggtggacagcaccgacaaggcggacctgcggctgatctacctggccctggcgcacatgatcaagttccgcggccacttcctgatcgagggcgacctgaacccggacaactcggacgtggacaagctgttcatccagctggtgcagacctacaaccagctgttcgaggagaaccccatcaacgcctccggcgtggacgccaaggcgatcctgtcggcgcgcctgtccaagtcgcggcgcctggagaacctgatcgcccagctgccgggcgagaagaagaacggcctgttcggcaacctgatcgcgctgagcctgggcctgacgcccaacttcaagtccaacttcgacctggccgaggacgcgaagctgcagctgtcgaaggacacctacgacgacgacctggacaacctgctggcccagatcggcgaccagtacgcggacctgttcctggccgccaagaacctgagcgacgccatcctgctgtccgacatcctgcgggtcaacaccgagatcacgaaggccccgctgagcgcgtccatgatcaagcggtacgacgagcaccaccaggacctgaccctgctgaaggcgctggtgcgccagcagctgcccgagaagtacaaggaaatcttcttcgaccagtcgaagaacggctacgccggctacatcgacggcggcgcgagccaggaggagttctacaagttcatcaagccgatcctggagaagatggacggcacggaggagctgctggtcaagctgaaccgcgaggacctgctgcgcaagcagcggaccttcgacaacggctcgatcccgcaccagatccacctgggcgagctgcacgccatcctgcggcgccaggaggacttctaccccttcctgaaggacaaccgcgagaagatcgagaagatcctgaccttccgcatcccgtactacgtgggccccctggcccgcggcaactcgcggttcgcgtggatgacccggaagagcgaggagaccatcacgccgtggaacttcgaggaggtcgtggacaagggcgcctcggcgcagagcttcatcgagcgcatgaccaacttcgacaagaacctgccgaacgagaaggtcctgcccaagcacagcctgctgtacgagtacttcaccgtgtacaacgagctgacgaaggtcaagtacgtgaccgagggcatgcggaagccggccttcctgtcgggcgagcagaagaaggcgatcgtggacctgctgttcaagaccaaccgcaaggtcacggtgaagcagctgaaggaggactacttcaagaagatcgagtgtttcgactcggtcgagatcagcggcgtggaggaccgcttcaacgccagcctgggcacctaccacgacctgctgaagatcatcaaggacaaggacttcctggacaacgaggagaacgaggacatcctggaggacatcgtcctgaccctgacgctgttcgaggaccgcgagatgatcgaggagcggctgaagacgtacgcccacctgttcgacgacaaggtgatgaagcagctgaagcggcgccgatacaccggctggggccgcctgtcgcggaagctgatcaacggcatccgggacaagcagtccggcaagaccatcctggacttcctgaagtcggacggcttcgcgaaccgcaacttcatgcagctgatccacgacgacagcctgaccttcaaggaggacatccagaaggcccaagtgagcggccagggcgactccctgcacgagcacatcgccaacctggcgggctcgccggcgatcaagaagggcatcctgcagaccgtcaaggtcgtggacgagctggtcaaggtgatgggccgccacaagcccgagaacatcgtgatcgagatggcccgggagaaccagaccacgcagaagggccagaagaacagccgcgagcggatgaagcgcatcgaggagggcatcaaggagctgggctcgcagatcctgaaggagcacccggtcgagaacacccagctgcagaacgagaagctgtacctgtactacctgcagaacggccgcgacatgtacgtggaccaggagctggacatcaaccggctgagcgactacgacgtggaccacatcgtgccgcagtcgttcctgaaggacgacagcatcgacaacaaggtcctgacccgctcggacaagaaccggggcaagtcggacaacgtgcccagcgaggaggtcgtgaagaagatgaagaactactggcgccagctgctgaacgccaagctgatcacgcagcgcaagttcgacaacctgaccaaggccgagcggggcggcctgagcgagctggacaaggcgggcttcatcaagcgccagctggtcgagacccggcagatcacgaagcacgtggcgcagatcctggactcgcggatgaacacgaagtacgacgagaacgacaagctgatccgcgaggtcaaggtgatcaccctgaagtccaagctggtctcggacttccgcaaggacttccagttctacaaggtccgggagatcaacaactaccaccacgcccacgacgcgtacctgaacgccgtcgtgggcaccgcgctgatcaagaagtacccgaagctggagtcggagttcgtctacggcgactacaaggtctacgacgtgcgcaagatgatcgccaagagcgagcaggagatcggcaaggccaccgcgaagtacttcttctactccaacatcatgaacttcttcaagaccgagatcacgctggccaacggcgagatccgcaagcgcccgctgatcgagaccaacggcgagacgggcgagatcgtctgggacaagggccgcgacttcgcgaccgtccggaaggtgctgagcatgccgcaggtcaacatcgtgaagaagaccgaggtgcagacgggcggcttctccaaggagtcgatcctgcccaagcgcaactcggacaagctgatcgcccggaagaaggactgggacccgaagaagtacggcggcttcgactcccccaccgtcgcctactcggtgctggtcgtggcgaaggtcgagaagggcaagtccaagaagctgaagtcggtgaaggagctgctgggcatcaccatcatggagcgctcgtcgttcgagaagaacccgatcgacttcctggaggcgaagggctacaaggaggtcaagaaggacctgatcatcaagctgcccaagtacagcctgttcgagctggagaacggccgcaagcggatgctggcctccgcgggcgagctgcagaagggcaacgagctggccctgccgtcgaagtacgtcaacttcctgtacctggcgtcgcactacgagaagctgaagggcagccccgaggacaacgagcagaagcagctgttcgtggagcagcacaagcactacctggacgagatcatcgagcagatcagcgagttctccaagcgggtcatcctggccgacgcgaacctggacaaggtgctgtcggcctacaacaagcaccgcgacaagccgatccgggagcaggcggagaacatcatccacctgttcaccctgacgaacctgggcgcccccgccgcgttcaagtacttcgacaccacgatcgaccgcaagcggtacacctccacgaaggaggtgctggacgcgaccctgatccaccagtcgatcaccggcctgtacgagacgcgcatcgacctgagccagctgggcggcgactcccgggcggacccgaagaagaagcggaaggtgtgatatttaattggggaccctagaggtcccctttatcgatgtcgacgtagttaacaaaggggacctctagggtccccagctggccagcgagtcatgaggtnaccatggtcattaggagccgctctcgcacttcagctgcttctccaagccgcagatgatcagctccaggccgaacaagaaggccggctcggcgccctggtggtcgaacagctcgatggcctggcgcagcaacggcggcatgctgtcggtggtcggggtctcgcgctcctccttggcgacctggtgctcctggtcctccaacacgcagcccagggtgaagtggcccacggccgacagggcgtacaacgcgttctccagcgagaagccctgctggcacaggaaggccaactggttctccagggtctcgtactgcttctcggtcggccgggtgcccaggtgcaccttggcgccgtcgcggtggctcagcaaggcgcagcggaagctcttggcgttgttgcgcaggaagtcctgccagctctcgccctccagcgggcagaagtgggtgtggtggcggtccaacatctcgatggccagggcgtcgagcagggcccgcttgttcttgacgtgccagtacagggtcggctgctcgacgcccagcttctgggccagcttgcgggtggtcaggccctcgatgccgacctcgttcagcagctccagggcggagttgatgaccttggacttgtccaggcgggacattgcgaagtgattcctcctgatgacgtcgtggcaggagggtcgcctgcgtcggcaactcgcccaggctacacgagagccctcgactgcgaaaatgccgaccaggcaccaccgcactccaggcttaacccggtgcgacgatccaatattacgagatctgatatcctcgaggcatgcgtcgacaactagcgtacgatcgactgccaggcatcaaataaaacgaaaggctcagtcgaaagactgggcctttcgttttatctgttgtttgtccggccatcatggccgcggtgatca

SEQ ID NO: 20 - DNA, 8423 bp, Escherichia coli
tcgcgcgtttcggtgatgacggtgaaaacctctgacacatgcagctcccggagacggtcacagcttgtctgtaagcggatgccgggagcagacaagcccgtcagggcgcgtcagcgggtgttggcgggtgtcggggctggcttaactatgcggcatcagagcagattgtactgagagtgcaccatatgcggtgtgaaataccgcacagatgcgtaaggagaaaataccgcatcaggcgccattcgccattcaggctgcgcaactgttgggaagggcgatcggtgcgggcctcttcgctattacgccagatcgagccgagaacgttatcgaagttggtcatgtgtaatcccctcgtttgaactttggattaagcgtagatacacccttggacaagccagttggattcggagacaagcaaattcagccttaaaaagggcgaggcctgcggggtggaacaccgcagggcctctaaccgctcgacgcgctgcaccaaccagcccgcgaacggctggcagccagcgtaaggcgcggctcatcgggcggcgttcgccacgatgtcctgcacttcgagccaagcctcgaacacctgctggtgtgcacgactcacccggttgttgacaccgcgcgcggccgtgcgggctcggtggggcggctgtgtcgcccttgccagcgtgagtagcgcgtacctcacctcgcccaacaggtcgcacacagccgattcgtacgccataaagccaggtgagcccaccagctccgtaagttcgggcgctgtgtggctcgtacccgcgcattcaggcggcagggggtctaacgggtctaaggcggcgtgtacggccgccacagcggctctcagcggcccggaaacgtcctcgaaacgacgcatgtgttcctcctggttggtacaggtggttgggggtgctcggctgtcgctggtgttccaccaccagggctcgacgggagagcgggggagtgtgcagttgtggggtggcccctcagcgaaatatctgacttggagctcgtgtcggaccatacaccggtgattaatcgtggtctactaccaagcgtgagccacgtcgccgacgaatttgagcagctctggctgccgtactggccgctggcaagcgacgatctgctcgaggggatctaccgccaaagccgcgcgtcggccctaggccgccggtacatcgaggcgaacccaacagcgctggcaaacctgctggtcgtggacgtagaccatccagacgcagcgctccgagcgctcagcgcccgggggtcccatccgctgcccaacgcgatcgtgggcaatcgcgccaacggccacgcacacgcagtgtgggcactcaacgcccctgttccacgcaccgaatacgcgcggcgtaagccgctcgcatacatggcggcgtgcgccgaaggccttcggcgcgccgtcgacggcgaccgcagttactcaggcctcatgaccaaaaaccccggccacatcgcctgggaaacggaatggctccactcagatctctacacactcagccacatcgaggccgagctcggcgcgaacatgccaccgccgcgctggcgtcagcagaccacgtacaaagcggctccgacgccgctagggcggaattgcgcactgttcgattccgtcaggttgtgggcctatcgtcccgccctcatgcggatctacctgccgacccggaacgtggacggactcggccgcgcgatctatgccgagtgccacgcgcgaaacgccgaattcccgtgcaacgacgtgtgtcccggaccgctaccggacagcgaggtccgcgccatcgccaacagcatttggcgttggatcacaaccaagtcgcgcatttgggcggacgggatcgtggtctacgaggccacactcagtgcgcgccagtcggccatctcgcggaagggcgcagcagcgcgcacggcggcgagcacagttgccggcgcgcaaagtccgcgtcagccatggaggcattgctatgagcgacggctacagcgacggctacagcgacggctacaaccggcagccgactgtccgcaaaagcggcgcgtgaccgccgccgaaggcgctcgaatcaccggactatccgaacgccacgtcgtccggctcgtggcgcaggaacgcagcgagtggctcgccgagcaggctgcacgccgcgaacgcatccgcgcctatcacgacgacgagggccactcttggccgcaaacggccaaacatttcgggctgcatctggacaccgttaagcgactcggctatcgggcgaggaaagagcgtgcggcagaacaggagcggctcaaaaggcccacaacgaagccgacaatccaccgctgttctaacgcaattggggagcgggtgtcgcgggggttccgtggggggttccgttgcaacgggtcggacaggtaaaagtcctggtagacgctagttttctggtttgggccatgcctgtctcgttgcgtgtttcgttgcgcccgttttgaataccagccagacgagacggggttctacgaatcttggtcgataccaagccatttccgctgaatatcggggagctcaccgccagaatcggtggttgtggtgatgtacgtggcgaactccgttgtagtgcctgtggtggcatccgtggccactctcgttgcacggttcgttgtgccgttacaggccccgttgacagctcaccgaacgtagttaaaacatgctggtcaaactaggtttaccaacgatacgagtcagctcatctagggccagttctaggcgttgttcgttgcgcggttcgttgcgcatgtttcgtgtggttgctagatggctccgcaaccacacgcttcgaggttgagtgcttccagcacgggcgcgatccagaagaacttcgtcgtgcgactgtcctcgttctgcattaatgaatcggccaacgcgcggggagaggcggtttgcgtattgggcgctcttccgcttcctcgctcactgactcgctgcgctcggtcgttcggctgcggcgagcggtatcagctcactcaaaggcggtaatacggttatccacagaatcaggggataacgcaggaaagaacatgtgagcaaaaggccagcaaaaggcaggaaccgtaaaaaggccgcgttgctggcgtttttccataggctccgcccccctgacgagcatcacaaaaatcgacgctcaagtcagaggtggcgaaacccgacaggactataaagataccaggcgtttccccctggaagctccctcgtgcgctctcctgttccgaccctgccgcttaccggatacctgtccgcctttctcccttcgggaagcgtggcgctttctcaatgctcacgctgtaggtatctcagttcggtgtaggtcgttcgctccaagctgggctgtgtgcacgaaccccccgttcagcccgaccgctgcgccttatccggtaactatcgtcttgagtccaacccggtaagacacgacttatcgccactggcagcagccactggtaacaggattagcagagcgaggtatgtaggcggtgctacagagttcttgaagtggtggcctaactacggctacactagaaggacagtatttggtatctgcgctctgctgaagccagttaccttcggaaaaagagttggtagctcttgatccggcaaacaaaccaccgctggtagcggtggtttttttgtttgcaagcagcagattacgcgcagaaaaaaaggatctcaagaagatcctttgatcttttctacggggtctgacgctcagtggaacgaaaactcacgttaagggattttggtcatgagattatcaaaaaggatcttcacctagatccttttaaattaaaaatgaagttttaaatcaatctaaagtatatatgagtaaacttggtctgacagttaccaatgcttaatcagtgaggcacctatctcagcgatctgtctatttcgttcatccatagttgcctgactccccgtcgtgtagataactacgatacgggagggcttaccatctggccccagtgctgcaatgataccgcgagacccacgctcaccggctccagatttatcagcaataaaccagccagccggaagggccgagcgcagagtggtcctgcaactttatccgcctccatccagtctattaattgttgccgggaagctagagtaagtagttcgccagttaatagtttgcgcaacgttgttgccattgctacaggcatcgtggtgtcacgctcgtcgtttggtatggcttcattcagctccggttcccaacgatcaaggcgagttacatgatcccccatgttgtgcaaaaaagcggttagctccttcggtcctccgatcgttgtcagaagtaagttggccgcagtgttatcactcatggttatggcagcactgcataattctcttactgtcatgccatccgtaagatgcttttctgtgactggtgagttcgagctgcagtgggatgaccttttaatgacctttaatagattatattactaattaattggggaccctagaggtccccttttttattttaaaaattttttcacaaaacggtttacaagcataaagctagtactgggcccgcggatccgatcccgtgacaaggccgaagagcccgcgaccgtgcggtcgtcgacgaccgagtgtgagcagaccccctggtgaagggtgaatcgacaggtacacacagccgccatacacttcgcttcatgcccttacggggggcggccaacccagaaggagattctcaatgggtaccaacggcgaccgcctctatcgggccgactcgcgtccgccggatgagatcaaacggtccggcggtctgatgccgcgtggccacaacgagtacttcgaccgcggtacgcagatgaacatcaatctgtacgaccacgcccgtgggacgcagaccggcttcgtccgctatgacgacggttacgtgtcgaccaagctgagcctgcgctcggcccatctggccggacaatccatcctgtccggctactccacgtactacatctacgtgattgcgaccgccccaaacatgttcaatgtgaacgacgtcctgggcgtctacagcccccatccctatgagcaggaagtgagcgccctcggcgggattccctatagccagatctacggttggtatcgggtcaactttggagtgatcgacgagcgcttgcaccggaaccgtgaatatcgcgatcggtactaccgcaacctgaacatcgcgccagcggaagatggctaccgcttggccgggttcccaccggaccaccaagcgtggcgggaggagccgtggattcaccacgcgccacagggctgtggcaattcctcgcggaccattaccggggacacctgcaacgaggaaacgcagaacctcagcacgatctatttgcgggagtaccagtcgaaggtgaagcgccaaatcttctcggactaccagtcggaggtcgacatctacaaccgcatccgggatgaactgtgagcggccgcgaaggagaagtaccggtgaacgcgcatccggccgggcccaggcacgccgaggaactgcaccacgcggatgtgcccgacaagccgcagagcccggacgagatcatgctgctggccccgaacgtgtggccgcgcaacctggttcgcggtgccgacggggtggtgacgatcgccggggtgccggtgaccgacctggccgcgaagttcggcacaccgctgttcgtgatcgacgaggacgacttccgcacccgctgccgcgacatcgccgcggcgttcggcggcggccagtacgtgcactacgcggccaaggcgttcctgtgctcggagatcgcgcgctgggtcgacgaggaaggcctgtccctcgacgtcgcgaccgggggagaactggccgtcgcgctgcacgccggcttcccggcctcgcggatcacggtgcacggcaacaacaaatccgtcgccgaactgaccgccgcggtgcaggcaggcgtgggccacgtcgtgctggactccgagatcgagatcgagcgcctcgatcagatcgccggtgcggcaggcgtggtccaggacgtgctggtgcgcgtcaccgtgggcgtggaggcccacacccacgagttcatctcgaccgcgcacgaggatcagaagttcggtttgtcgctggccacgggtgcggcgatgaacgcgatccgccgggtcttcgcgaccgacaacctgcgcctggtgggcctgcacagccacatcggctcgcagatcttcgacgtcgccgggttcgagatcgccgcgcaccgcgtgatcggcctgctgcgcgacgtggtcgccgagttcggcgtggagaagacctcgcagatgtccatcgtggatctcggtgggggactgggtatctcgtacctgccgcacgacgatccgccgcccatgaaggaactggccgacaagctgctggagatcgtgcgcaccgagtcggccgcggtcgggctgcccacgcccaagctcgtggtggaacccggacgcgccatcgcgggcccgggcaccatcacgctctacgaggtcggcacggtcaaggacgtggccgtcagccagaccgcgcaccgccgttacgtcagcgtcgacggcggcatgagcgacaacatccgcacgtcgctgtacgccgcgcagtacgacgcccggttggtgtcacgcgtcagcgacgctccgcccgcactggcgcggatcgtcggaaaacactgtgagagtggcgatatcgtcgtccgcgacacctgggtgtccgacgacatcgcgcccggcgacctgatcggtgtcgccgcgaccggcgcgtactgctactcgatgtcgagtcgatacaacctgctgtgccgccccgctgtggtggccgtcgccgacggccaggcacgtctggtgctgcgacgggagaccgtcgaggatcttctgagcctggaggtgaagggtcaatgagcggccgccagctgagcgccggtcgctaccattaccagttggtctggtgtcaaaaataataataaccgggcaggccatgtctgcccgtatttcgcgtaaggaaatccattatgtactatttgacctgcagggggggggggcgctgaggtctgcctcgtgaagaaggtgttgctgactcataccaggcctgaatcgccccatcatccagccagaaagtgagggagccacggttgatgagagctttgttgtaggtggaccagttggtgattttgaacttttgctttgccacggaacggtctgcgttgtcgggaagatgcgtgatctgatccttcaactcagcaaaagttcgatttattcaacaaagccgccgtcccgtcaagtcagcgtaatgctctgccagtgttacaaccaattaaccaattctgattagaaaaactcatcgagcatcaaatgaaactgcaatttattcatatcaggattatcaataccatatttttgaaaaagccgtttctgtaatgaaggagaaaactcaccgaggcagttccataggatggcaagatcctggtatcggtctgcgattccgactcgtccaacatcaatacaacctattaatttcccctcgtcaaaaataaggttatcaagtgagaaatcaccatgagtgacgactgaatccggtgagaatggcaaaagcttatgcatcatcaggagtacggataaaatgcttgatggtcggaagaggcataaattccgtcagccagtttagtctgaccatctcatctgtaacatcattggcaacgctacctttgccatgtttcagaaacaactctggcgcatcgggcttcccatacaatcgatagattgtcgcacctgattgcccgacattatcgcgagcccatttatacccatataaatcagcatccatgttggaatttaatcgcggcctcgagcaagacgtttcccgttgaatatggctcataacaccccttgtattactgtttatgtaagcagacagttttattgttcatgatgatatatttttatcttgtgcaatgtaacatcagagattttgagacacaacgtggctttgttgaataaatcgaacttttgctgagttgaaggatcagatcacgcatcttcccgacaacgcagaccgttccgtggcaaagcaaaagttcaaaatcaccaactggtccacctacaacaaagctctcatcaaccgtggctccctcactttctggctggatgatggggcgattcaggcctggtatgagtcagcaacaccttcttcacgaggcagacctcagcgctgcaggtcattattgaagcatttatcagggttattgtctcatgagcggatacatatttgaatgtatttagaaaaataaacaaataggggttccgcgcacatttccccgaaaagtgccacctgacgtctaagaaaccattattatcatgacattaacctataaaaataggcgtatcacgaggccctttcgtc

SEQ ID NO: 21 - DNA, 8026 bp, Escherichia coli
tcgcgcgtttcggtgatgacggtgaaaacctctgacacatgcagctcccggagacggtcacagcttgtctgtaagcggatgccgggagcagacaagcccgtcagggcgcgtcagcgggtgttggcgggtgtcggggctggcttaactatgcggcatcagagcagattgtactgagagtgcaccatatgcggtgtgaaataccgcacagatgcgtaaggagaaaataccgcatcaggcgccattcgccattcaggctgcgcaactgttgggaagggcgatcggtgcgggcctcttcgctattacgccagatcgagccgagaacgttatcgaagttggtcatgtgtaatcccctcgtttgaactttggattaagcgtagatacacccttggacaagccagttggattcggagacaagcaaattcagccttaaaaagggcgaggcctgcggggtggaacaccgcagggcctctaaccgctcgacgcgctgcaccaaccagcccgcgaacggctggcagccagcgtaaggcgcggctcatcgggcggcgttcgccacgatgtcctgcacttcgagccaagcctcgaacacctgctggtgtgcacgactcacccggttgttgacaccgcgcgcggccgtgcgggctcggtggggcggctgtgtcgcccttgccagcgtgagtagcgcgtacctcacctcgcccaacaggtcgcacacagccgattcgtacgccataaagccaggtgagcccaccagctccgtaagttcgggcgctgtgtggctcgtacccgcgcattcaggcggcagggggtctaacgggtctaaggcggcgtgtacggccgccacagcggctctcagcggcccggaaacgtcctcgaaacgacgcatgtgttcctcctggttggtacaggtggttgggggtgctcggctgtcgctggtgttccaccaccagggctcgacgggagagcgggggagtgtgcagttgtggggtggcccctcagcgaaatatctgacttggagctcgtgtcggaccatacaccggtgattaatcgtggtctactaccaagcgtgagccacgtcgccgacgaatttgagcagctctggctgccgtactggccgctggcaagcgacgatctgctcgaggggatctaccgccaaagccgcgcgtcggccctaggccgccggtacatcgaggcgaacccaacagcgctggcaaacctgctggtcgtggacgtagaccatccagacgcagcgctccgagcgctcagcgcccgggggtcccatccgctgcccaacgcgatcgtgggcaatcgcgccaacggccacgcacacgcagtgtgggcactcaacgcccctgttccacgcaccgaatacgcgcggcgtaagccgctcgcatacatggcggcgtgcgccgaaggccttcggcgcgccgtcgacggcgaccgcagttactcaggcctcatgaccaaaaaccccggccacatcgcctgggaaacggaatggctccactcagatctctacacactcagccacatcgaggccgagctcggcgcgaacatgccaccgccgcgctggcgtcagcagaccacgtacaaagcggctccgacgccgctagggcggaattgcgcactgttcgattccgtcaggttgtgggcctatcgtcccgccctcatgcggatctacctgccgacccggaacgtggacggactcggccgcgcgatctatgccgagtgccacgcgcgaaacgccgaattcccgtgcaacgacgtgtgtcccggaccgctaccggacagcgaggtccgcgccatcgccaacagcatttggcgttggatcacaaccaagtcgcgcatttgggcggacgggatcgtggtctacgaggccacactcagtgcgcgccagtcggccatctcgcggaagggcgcagcagcgcgcacggcggcgagcacagttgccggcgcgcaaagtccgcgtcagccatggaggcattgctatgagcgacggctacagcgacggctacagcgacggctacaaccggcagccgactgtccgcaaaagcggcgcgtgaccgccgccgaaggcgctcgaatcaccggactatccgaacgccacgtcgtccggctcgtggcgcaggaacgcagcgagtggctcgccgagcaggctgcacgccgcgaacgcatccgcgcctatcacgacgacgagggccactcttggccgcaaacggccaaacatttcgggctgcatctggacaccgttaagcgactcggctatcgggcgaggaaagagcgtgcggcagaacaggagcggctcaaaaggcccacaacgaagccgacaatccaccgctgttctaacgcaattggggagcgggtgtcgcgggggttccgtggggggttccgttgcaacgggtcggacaggtaaaagtcctggtagacgctagttttctggtttgggccatgcctgtctcgttgcgtgtttcgttgcgcccgttttgaataccagccagacgagacggggttctacgaatcttggtcgataccaagccatttccgctgaatatcggggagctcaccgccagaatcggtggttgtggtgatgtacgtggcgaactccgttgtagtgcctgtggtggcatccgtggccactctcgttgcacggttcgttgtgccgttacaggccccgttgacagctcaccgaacgtagttaaaacatgctggtcaaactaggtttaccaacgatacgagtcagctcatctagggccagttctaggcgttgttcgttgcgcggttcgttgcgcatgtttcgtgtggttgctagatggctccgcaaccacacgcttcgaggttgagtgcttccagcacgggcgcgatccagaagaacttcgtcgtgcgactgtcctcgttctgcattaatgaatcggccaacgcgcggggagaggcggtttgcgtattgggcgctcttccgcttcctcgctcactgactcgctgcgctcggtcgttcggctgcggcgagcggtatcagctcactcaaaggcggtaatacggttatccacagaatcaggggataacgcaggaaagaacatgtgagcaaaaggccagcaaaaggcaggaaccgtaaaaaggccgcgttgctggcgtttttccataggctccgcccccctgacgagcatcacaaaaatcgacgctcaagtcagaggtggcgaaacccgacaggactataaagataccaggcgtttccccctggaagctccctcgtgcgctctcctgttccgaccctgccgcttaccggatacctgtccgcctttctcccttcgggaagcgtggcgctttctcaatgctcacgctgtaggtatctcagttcggtgtaggtcgttcgctccaagctgggctgtgtgcacgaaccccccgttcagcccgaccgctgcgccttatccggtaactatcgtcttgagtccaacccggtaagacacgacttatcgccactggcagcagccactggtaacaggattagcagagcgaggtatgtaggcggtgctacagagttcttgaagtggtggcctaactacggctacactagaaggacagtatttggtatctgcgctctgctgaagccagttaccttcggaaaaagagttggtagctcttgatccggcaaacaaaccaccgctggtagcggtggtttttttgtttgcaagcagcagattacgcgcagaaaaaaaggatctcaagaagatcctttgatcttttctacggggtctgacgctcagtggaacgaaaactcacgttaagggattttggtcatgagattatcaaaaaggatcttcacctagatccttttaaattaaaaatgaagttttaaatcaatctaaagtatatatgagtaaacttggtctgacagttaccaatgcttaatcagtgaggcacctatctcagcgatctgtctatttcgttcatccatagttgcctgactccccgtcgtgtagataactacgatacgggagggcttaccatctggccccagtgctgcaatgataccgcgagacccacgctcaccggctccagatttatcagcaataaaccagccagccggaagggccgagcgcagagtggtcctgcaactttatccgcctccatccagtctattaattgttgccgggaagctagagtaagtagttcgccagttaatagtttgcgcaacgttgttgccattgctacaggcatcgtggtgtcacgctcgtcgtttggtatggcttcattcagctccggttcccaacgatcaaggcgagttacatgatcccccatgttgtgcaaaaaagcggttagctccttcggtcctccgatcgttgtcagaagtaagttggccgcagtgttatcactcatggttatggcagcactgcataattctcttactgtcatgccatccgtaagatgcttttctgtgactggtgagttcgagctgcagtgggatgaccttttaatgacctttaatagattatattactaattaattggggaccctagaggtccccttttttattttaaaaattttttcacaaaacggtttacaagcataaagctagtactgggcccgcggatccgatcccgtgacaaggccgaagagcccgcgaccgtgcggtcgtcgacgaccgagtgtgagcagaccccctggtgaagggtgaatcgacaggtacacacagccgccatacacttcgcttcatgcccttacggggggcggccaacccagaaggagattctcaatgggtaccaacggcgaccgcctctatcgggccgactcgcgtccgccggatgagatcaaacggtccggcggtctgatgccgcgtggccacaacgagtacttcgaccgcggtacgcagatgaacatcaatctgtacgaccacgcccgtgggacgcagaccggcttcgtccgctatgacgacggttacgtgtcgaccaagctgagcctgcgctcggcccatctggccggacaatccatcctgtccggctactccacgtactacatctacgtgattgcgaccgccccaaacatgttcaatgtgaacgacgtcctgggcgtctacagcccccatccctatgagcaggaagtgagcgccctcggcgggattccctatagccagatctacggttggtatcgggtcaactttggagtgatcgacgagcgcttgcaccggaaccgtgaatatcgcgatcggtactaccgcaacctgaacatcgcgccagcggaagatggctaccgcttggccgggttcccaccggaccaccaagcgtggcgggaggagccgtggattcaccacgcgccacagggctgtggcaattcctcgcggaccattaccggggacacctgcaacgaggaaacgcagaacctcagcacgatctatttgcgggagtaccagtcgaaggtgaagcgccaaatcttctcggactaccagtcggaggtcgacatctacaaccgcatccgggatgaactgtgagcggccgcggtaccagatctttaaatctagaggtgaccacaacgacgcgcccgctttgatcggggacgtctgcggccgaccatttacgggtcttgttgtcgttggcggtcatgggccgaacatactcacccggatcggagggccgaggacaaggtcgaacgaggggcatgacccggtgcggggcttcttgcactcggcataggcgagtgctaagaataacgttggcactcgcgaccggtgagtcgtaggtcgggacggtgaggccaggcccgtcgtcgcagcgagtggcagcgaggacaacttgagccgtccgtcgcgggcactgcgcccggccagcgtaagtagcggggttgccgtcacccggtgacccccggtttcatccccgatccggaggaatcacttcgcaatggccaagacaattgcggatccacatagctgaattctaactaactgacggagcgaatgtgaacgcgcatccggccgggcccaggcacgccgaggaactgcaccacgcggatgtgcccgacaagccgcagagcccggacgagatcatgctgctggccccgaacgtgtggccgcgcaacctggttcgcggtgccgacggggtggtgacgatcgccggggtgccggtgaccgacctggccgcgaagttcggcacaccgctgttcgtgatcgacgaggacgacttccgcacccgctgccgcgacatcgccgcggcgttcggcggcggccagtacgtgcactacgcggccaaggcgttcctgtgctcggagatcgcgcgctgggtcgacgaggaaggcctgtccctcgacgtcgcgaccgggggagaactggccgtcgcgctgcacgccggcttcccggcctcgcggatcacggtgcacggcaacaacaaatccgtcgccgaactgaccgccgcggtgcaggcaggcgtgggccacgtcgtgctggactccgagatcgagatcgagcgcctcgatcagatcgccggtgcggcaggcgtggtccaggacgtgctggtgcgcgtcaccgtgggcgtggaggcccacacccacgagttcatctcgaccgcgcacgaggatcagaagttcggtttgtcgctggccacgggtgcggcgatgaacgcgatccgccgggtcttcgcgaccgacaacctgcgcctggtgggcctgcacagccacatcggctcgcagatcttcgacgtcgccgggttcgagatcgccgcgcaccgcgtgatcggcctgctgcgcgacgtggtcgccgagttcggcgtggagaagacctcgcagatgtccatcgtggatctcggtgggggactgggtatctcgtacctgccgcacgacgatccgccgcccatgaaggaactggccgacaagctgctggagatcgtgcgcaccgagtcggccgcggtcgggctgcccacgcccaagctcgtggtggaacccggacgcgccatcgcgggcccgggcaccatcacgctctacgaggtcggcacggtcaaggacgtggccgtcagccagaccgcgcaccgccgttacgtcagcgtcgacggcggcatgagcgacaacatccgcacgtcgctgtacgccgcgcagtacgacgcccggttggtgtcacgcgtcagcgacgctccgcccgcactggcgcggatcgtcggaaaacactgtgagagtggcgatatcgtcgtccgcgacacctgggtgtccgacgacatcgcgcccggcgacctgatcggtgtcgccgcgaccggcgcgtactgctactcgatgtcgagtcgatacaacctgctgtgccgccccgctgtggtggccgtcgccgacggccaggcacgtctggtgctgcgacgggagaccgtcgaggatcttctgagcctggaggtgaagggtcaatgagtaagaagcccatcgatagattgtcgcacctgattgcccgacattatcgcgagcccatttatacccatataaatcagcatccatgttggaatttaatcgcggcctcgagcaagacgtttcccgttgaatatggctcataacaccccttgtattactgtttatgtaagcagacagttttattgttcatgatgatatatttttatcttgtgcaatgtaacatcagagattttgagacacaacgtggctttgttgaataaatcgaacttttgctgagttgaaggatcagatcacgcatcttcccgacaacgcagaccgttccgtggcaaagcaaaagttcaaaatcaccaactggtccacctacaacaaagctctcatcaaccgtggctccctcactttctggctggatgatggggcgattcaggcctggtatgagtcagcaacaccttcttcacgaggcagacctcagcgctgcaggtcattattgaagcatttatcagggttattgtctcatgagcggatacatatttgaatgtatttagaaaaataaacaaataggggttccgcgcacatttccccgaaaagtgccacctgacgtctaagaaaccattattatcatgacattaacctataaaaataggcgtatcacgaggccctttcgtc